European Patent Application EP 4 516 809 A2, published March 5, 2025. Title: Bispecific Antibodies specifically binding to PD1 and LAG3. Applicant: F. Hoffmann-La Roche AG. Application EP PCT/EP2018/058382, filed April 3, 2018. The sequence listing filed with the application follows.

SEQUENCE LISTING (169 sequences)

SEQ ID NO: 1 - protein, 7 aa, synthetic construct
  REGION 1..7: note = heavy chain HVR-H1, PD1-0103
GFSFSSY

SEQ ID NO: 2 - skipped

SEQ ID NO: 3 - protein, 9 aa, synthetic construct
  REGION 1..9: note = heavy chain HVR-H3, PD1-0103
TGRVYFALD

SEQ ID NO: 4 - protein, 11 aa, synthetic construct
  REGION 1..11: note = light chain HVR-L1, PD1-0103
SESVDTSDNSF

SEQ ID NO: 5 - skipped

SEQ ID NO: 6 - protein, 6 aa, synthetic construct
  REGION 1..6: note = light chain HVR-L3, PD1-0103
NYDVPW

SEQ ID NO: 7 - protein, 120 aa, synthetic construct
  REGION 1..120: note = heavy chain variable domain VH, PD1-0103
EVILVESGGGLVKPGGSLKLSCAASGFSFSSYTMSWVRQTPEKRLDWVATISGGGRDIYYPDSVKGRFTISRDNAKNTLYLEMSSLMSEDTALYYCVLLTGRVYFALDSWGQGTSVTVSS

SEQ ID NO: 8 - protein, 111 aa, synthetic construct
  REGION 1..111: note = light chain variable domain VL, PD1-0103
KIVLTQSPASLPVSLGQRATISCRASESVDTSDNSFIHWYQQRPGQSPKLLIYRSSTLESGVPARFSGSGSRTDFTLTIDPVEADDVATYYCQQNYDVPWTFGGGTKLEIK

SEQ ID NO: 9 - protein, 120 aa, synthetic construct
  REGION 1..120: note = humanized variant -heavy chain variable domain VH of PD1-0103_01 (PD1 0376)
EVQLLESGGGLVQPGGSLRLSCAASGFSFSSYTMSWVRQAPGKGLEWVATISGGGRDIYYPDSVKGRFTISRDNSKNTLYLQMNSLRAEDTAVYYCVLLTGRVYFALDSWGQGTLVTVSS

SEQ ID NO: 10 - protein, 111 aa, synthetic construct
  REGION 1..111: note = humanized variant -light chain variable domain VL of PD1-0103_01 (PD1 0376)
DIVMTQSPDSLAVSLGERATINCKASESVDTSDNSFIHWYQQKPGQSPKLLIYRSSTLESGVPDRFSGSGSGTDFTLTISSLQAEDVAVYYCQQNYDVPWTFGQGTKVEIK

SEQ ID NO: 11 - protein, 111 aa, synthetic construct
  REGION 1..111: note = humanized variant -light chain variable domain VL of PD1-0103_02
DVVMTQSPLSLPVTLGQPASISCRASESVDTSDNSFIHWYQQRPGQSPRLLIYRSSTLESGVPDRFSGSGSGTDFTLKISRVEAEDVGVYYCQQNYDVPWTFGQGTKVEIK

SEQ ID NO: 12 - protein, 111 aa, synthetic construct
  REGION 1..111: note = humanized variant -light chain variable domain VL of PD1-0103_03
EIVLTQSPATLSLSPGERATLSCRASESVDTSDNSFIHWYQQKPGQSPRLLIYRSSTLESGIPARFSGSGSGTDFTLTISSLEPEDFAVYYCQQNYDVPWTFGQGTKVEIK

SEQ ID NO: 13 - protein, 111 aa, synthetic construct; identical to SEQ ID NO: 12
  REGION 1..111: note = humanized variant -light chain variable domain VL of PD1-0103_04

SEQ ID NO: 14 - protein, 5 aa, synthetic construct
  REGION 1..5: note = heavy chain HVR-H1, aLAG3(0414)
DYTMN

SEQ ID NO: 15 - protein, 17 aa, synthetic construct
  REGION 1..17: note = heavy chain HVR-H2, aLAG3(0414)
VISWDGGGTYYTDSVKG

SEQ ID NO: 16 - protein, 12 aa, synthetic construct
  REGION 1..12: note = heavy chain HVR-H3, aLAG3(0414)
GLTDTTLYGSDY

SEQ ID NO: 17 - protein, 11 aa, synthetic construct
  REGION 1..11: note = light chain HVR-L1, aLAG3(0414)
RASQSISSYLN

SEQ ID NO: 18 - protein, 7 aa, synthetic construct
  REGION 1..7: note = light chain HVR-L2, aLAG3(0414)
AASTLQS

SEQ ID NO: 19 - protein, 9 aa, synthetic construct
  REGION 1..9: note = light chain HVR-L3, aLAG3(0414)
QQTYSSPLT

SEQ ID NO: 20 - protein, 121 aa, synthetic construct
  REGION 1..121: note = heavy chain variable domain VH, aLAG3(0414)
EVQLLESGGGLVQPGGSLRLSCAASGFIFDDYTMNWVRQAPGKGLEWVAVISWDGGGTYYTDSVKGRFTISRDDFKNTLYLQMNSLRAEDTAVYYCAKGLTDTTLYGSDYWGQGTLVTVSS

SEQ ID NO: 21 - protein, 107 aa, synthetic construct
  REGION 1..107: note = light chain variable domain VL, aLAG3(0414)
DIQMTQSPSSLSASVGDRVTITCRASQSISSYLNWYQQKPGKAPKLLIYAASTLQSGVPSRFSGSGSGTDFTLTISSLQPEDFATYYCQQTYSSPLTFGGGTKVEIK

SEQ ID NO: 22 - protein, 5 aa, synthetic construct
  REGION 1..5: note = heavy chain HVR-H1, aLAG3(0403)
DYTMH

SEQ ID NO: 23 - protein, 17 aa, synthetic construct
  REGION 1..17: note = heavy chain HVR-H2, aLAG3(0403)
LVSWDGGGTYYTNSVKG

SEQ ID NO: 24 - protein, 12 aa, synthetic construct
  REGION 1..12: note = heavy chain HVR-H3, aLAG3(0403)
AITDTSLYGYDY

SEQ ID NO: 25 - protein, 11 aa, synthetic construct
  REGION 1..11: note = light chain HVR-L1, aLAG3(0403)
RASQSISSYLN

SEQ ID NO: 26 - protein, 7 aa, synthetic construct
  REGION 1..7: note = light chain HVR-L2, aLAG3(0403)
AASSLQS

SEQ ID NO: 27 - protein, 9 aa, synthetic construct
  REGION 1..9: note = light chain HVR-L3, aLAG3(0403)
QQTYSTPLT

SEQ ID NO: 28 - protein, 121 aa, synthetic construct
  REGION 1..121: note = heavy chain variable domain VH, aLAG3(0403)
EVQLLESGGGLVQPGGSLRLSCAASGFTFDDYTMHWVRQAPGKGLEWVSLVSWDGGGTYYTNSVKGRFTISRDNSKNTLYLQMNSLRAEDTAVYFCAKAITDTSLYGYDYWGQGILVTVSS

SEQ ID NO: 29 - protein, 107 aa, synthetic construct
  REGION 1..107: note = light chain variable domain VL, aLAG3(0403)
DIQMTQSPSSLSASVGDRVTITCRASQSISSYLNWYQQKPGNAPKLLIYAASSLQSGVPSRFSGSGSGTDFTLTISSLQPEDFATYYCQQTYSTPLTFGGGTKVEIK

SEQ ID NO: 30 - protein, 5 aa, synthetic construct
  REGION 1..5: note = heavy chain HVR-H1, aLAG3(0411)
DYTMN

SEQ ID NO: 31 - protein, 17 aa, synthetic construct
  REGION 1..17: note = heavy chain HVR-H2, aLAG3(0411)
VISWDGGATYYADSVKG

SEQ ID NO: 32 - protein, 12 aa, synthetic construct
  REGION 1..12: note = heavy chain HVR-H3, aLAG3(0411)
GLTDDTLYGSDY

SEQ ID NO: 33 - protein, 11 aa, synthetic construct
  REGION 1..11: note = light chain HVR-L1, aLAG3(0411)
RASQSIVSYLN

SEQ ID NO: 34 - protein, 7 aa, synthetic construct
  REGION 1..7: note = light chain HVR-L2, aLAG3(0411)
ASSSLQS

SEQ ID NO: 35 - protein, 9 aa, synthetic construct
  REGION 1..9: note = light chain HVR-L3, aLAG3(0411)
QQTYSTPLT

SEQ ID NO: 36 - protein, 121 aa, synthetic construct
  REGION 1..121: note = heavy chain variable domain VH, aLAG3(0411)
EVHLLESGGGLVQPGGSLRLSCAASGFIVDDYTMNWVRQAPGKGLEWVSVISWDGGATYYADSVKGRFTISRDDFKNTLYLQMNSLRAEDTAVYYCAKGLTDDTLYGSDYWGQGTLVTVSS

SEQ ID NO: 37 - protein, 107 aa, synthetic construct
  REGION 1..107: note = light chain variable domain VL, aLAG3(0411)
DIQMTQSPSSLSASVGDRVTITCRASQSIVSYLNWYQQKPGKAPKLLIYASSSLQSGVPSRFSGSGSGTDFTLTISSLQPEDFATYYCQQTYSTPLTFGGGTKVEIK

SEQ ID NO: 38 - protein, 5 aa, synthetic construct
  REGION 1..5: note = heavy chain HVR-H1, aLAG3(0417)
DYAMS

SEQ ID NO: 39 - protein, 17 aa, synthetic construct
  REGION 1..17: note = heavy chain HVR-H2, aLAG3(0417)
GIDNSGYYTYYTDSVKG

SEQ ID NO: 40 - protein, 13 aa, synthetic construct
  REGION 1..13: note = heavy chain HVR-H3, aLAG3(0417)
THSGLIVNDAFDI

SEQ ID NO: 41 - protein, 11 aa, synthetic construct
  REGION 1..11: note = light chain HVR-L1, aLAG3(0417)
RASQSISSYLN

SEQ ID NO: 42 - protein, 7 aa, synthetic construct
  REGION 1..7: note = light chain HVR-L2, aLAG3(0417)
AASSLQS

SEQ ID NO: 43 - protein, 9 aa, synthetic construct
  REGION 1..9: note = light chain HVR-L3, aLAG3(0417)
QQTYSTPLT

SEQ ID NO: 44 - protein, 122 aa, synthetic construct
  REGION 1..122: note = heavy chain variable domain VH, aLAG3(0417)
EVQLVESGGGLVQPGGSLRLACAASGFTFSDYAMSWVRQAPGKGLEWVSGIDNSGYYTYYTDSVKGRFTISRDDVKNTLYLQMNSLRAEDTAVYLCTKTHSGLIVNDAFDIWGQGTMVTVSS

SEQ ID NO: 45 - protein, 107 aa, synthetic construct
  REGION 1..107: note = light chain variable domain VL, aLAG3(0417)
DIQMTQSPSSLSASVGDRVTITCRASQSISSYLNWYQQKPGKAPKLLIYAASSLQSGVPSRFSGSGSGTDFTLTISSLQPEDFATYYCQQTYSTPLTFGGGTKVEIK

SEQ ID NO: 46 - protein, 5 aa, synthetic construct
  REGION 1..5: note = heavy chain HVR-H1, aLAG3(0416)
DYAMS

SEQ ID NO: 47 - protein, 17 aa, synthetic construct
  REGION 1..17: note = heavy chain HVR-H2, aLAG3(0416)
GIDNSGYYTYYTDSVKG

SEQ ID NO: 48 - protein, 13 aa, synthetic construct
  REGION 1..13: note = heavy chain HVR-H3, aLAG3(0416)
THSGLIVNDAFDI

SEQ ID NO: 49 - protein, 11 aa, synthetic construct
  REGION 1..11: note = light chain HVR-L1, aLAG3(0416)
RASQSISSYLN

SEQ ID NO: 50 - protein, 7 aa, synthetic construct
  REGION 1..7: note = light chain HVR-L2, aLAG3(0416)
DASSLES

SEQ ID NO: 51 - protein, 9 aa, synthetic construct
  REGION 1..9: note = light chain HVR-L3, aLAG3(0416)
QQSYSTPLT

SEQ ID NO: 52 - protein, 122 aa, synthetic construct; identical to SEQ ID NO: 44
  REGION 1..122: note = heavy chain variable domain VH, aLAG3(0416)

SEQ ID NO: 53 - protein, 107 aa, synthetic construct
  REGION 1..107: note = light chain variable domain VL, aLAG3(0416)
DIQLTQSPSSLSASVGDRVTITCRASQSISSYLNWYQQKPGKAPKLLIYDASSLESGVPSRFSGSGSGTDATLTISSLQPEDFATYYCQQSYSTPLTFGGGTKVEIK

SEQ ID NO: 54 - protein, 120 aa, synthetic construct
  REGION 1..120: note = heavy chain variable domain VH, BMS-986016
QVQLQQWGAGLLKPSETLSLTCAVYGGSFSDYYWNWIRQPPGKGLEWIGEINHRGSTNSNPSLKSRVTLSLDTSKNQFSLKLRSVTAADTAVYYCAFGYSDYEYNWFDPWGQGTLVTVSS

SEQ ID NO: 55 - protein, 107 aa, synthetic construct
  REGION 1..107: note = light chain variable domain VL BMS-986016
EIVLTQSPATLSLSPGERATLSCRASQSISSYLAWYQQKPGQAPRLLIYDASNRATGIPARFSGSGSGTDFTLTISSLEPEDFAVYYCQQRSNWPLTFGQGTNLEIK

SEQ ID NO: 56 - protein, 5 aa, synthetic construct
  REGION 1..5: note = heavy chain HVR-H1, MDX25F7 (25F7)
DYYWN

SEQ ID NO: 57 - protein, 16 aa, synthetic construct
  REGION 1..16: note = heavy chain HVR-H2, MDX25F7 (25F7)
EINHNGNTNSNPSLKS

SEQ ID NO: 58 - protein, 10 aa, synthetic construct
  REGION 1..10: note = heavy chain HVR-H3, MDX25F7 (25F7)
GYSDYEYNWF

SEQ ID NO: 59 - protein, 11 aa, synthetic construct
  REGION 1..11: note = light chain HVR-L1, MDX25F7 (25F7)
RASQSISSYLA

SEQ ID NO: 60 - protein, 7 aa, synthetic construct
  REGION 1..7: note = light chain HVR-L2, MDX25F7 (25F7)
DASNRAT

SEQ ID NO: 61 - protein, 9 aa, synthetic construct
  REGION 1..9: note = light chain HVR-L3, MDX25F7 (25F7)
QQRSNWPLT

SEQ ID NO: 62 - protein, 120 aa, synthetic construct
  REGION 1..120: note = heavy chain variable domain VH, MDX25F7 (25F7)
QVQLQQWGAGLLKPSETLSLTCAVYGGSFSDYYWNWIRQPPGKGLEWIGEINHNGNTNSNPSLKSRVTLSLDTSKNQFSLKLRSVTAADTAVYYCAFGYSDYEYNWFDPWGQGTLVTVSS

SEQ ID NO: 63 - protein, 107 aa, synthetic construct; identical to SEQ ID NO: 55
  REGION 1..107: note = light chain variable domain VL, MDX25F7 (25F7)

SEQ ID NO: 64 - protein, 125 aa, synthetic construct
  REGION 1..125: note = heavy chain variable domain VH, humanized BAP050 (LAG525)
QIQLVQSGPELKKPGETVKISCKASGFTLTNYGMNWVRQTPGKGLKWMGWINTDTGEPTYADDFKGRFAFSLETSASTASLQINNLKNADTATYFCARNPPYYYGTNNAEAMDYWGQGTTVTVSS

SEQ ID NO: 65 - protein, 107 aa, synthetic construct
  REGION 1..107: note = light chain variable domain VL, humanized BAP050 (LAG525)
DIQMTQTTSSLSASLGDRVTISCSSSQDISNYLMWYQQKPDGTVKVLIYYTSTLHLGVPSRFSGSGSGTDYSLTISNLELEDIATYYCQQYYNLPWTFGQGTKVEIK

SEQ ID NO: 66 - protein, 122 aa, synthetic construct
  REGION 1..122: note = heavy chain variable domain VH, MDX26H10 (26H10)
QVQLVESGGGVVQPGRSLRLSCAASGFTFSSYGMHWVRQAPGKGLEWVAVIWYDGSNKYYADSVKGRFTISRDNSKNTLYLQMNSLRAEDTAVYYCAREWAVASWDYGMDVWGQGTTVTVSS

SEQ ID NO: 67 - protein, 108 aa, synthetic construct
  REGION 1..108: note = light chain variable domain VL, MDX26H10 (26H10)
EIVLTQSPGTLSLSPGERATLSCRASQSVSSSYLAWYQQKPGQAPRLLIYGASSRATGIPDRFSGSGSGTDFTLTISRLEPEDFAVYYCQQYGSSPFTFGPGTKVDIK

SEQ ID NO: 68 - protein, 107 aa, synthetic construct [sequence omitted]

SEQ ID NO: 69 - protein, 105 aa, synthetic construct
  REGION 1..105: note = human lambda light chain constant region
QPKAAPSVTLFPPSSEELQANKATLVCLISDFYPGAVTVAWKADSSPVKAGVETTTPSKQSNNKYAASSYLSLTPEQWKSHRSYSCQVTHEGSTVEKTVAPTECS

SEQ ID NO: 70 - protein, 329 aa, synthetic construct
  REGION 1..329: note = human heavy chain constant region derived from IgG1
ASTKGPSVFPLAPSSKSTSGGTAALGCLVKDYFPEPVTVSWNSGALTSGVHTFPAVLQSSGLYSLSSVVTVPSSSLGTQTYICNVNHKPSNTKVDKKVEPKSCDKTHTCPPCPAPELLGGPSVFLFPPKPKDTLMISRTPEVTCVVVDVSHEDPEVKFNWYVDGVEVHNAKTKPREEQYNSTYRVVSVLTVLHQDWLNGKEYKCKVSNKALPAPIEKTISKAKGQPREPQVYTLPPSRDELTKNQVSLTCLVKGFYPSDIAVEWESNGQPENNYKTTPPVLDSDGSFFLYSKLTVDKSRWQQGNVFSCSVMHEALHNHYTQKSLSLSPG

SEQ ID NO: 71 - protein, 329 aa, synthetic construct
  REGION 1..329: note = human heavy chain constant region derived from IgG1 with mutations L234A, L235A and P329G
ASTKGPSVFPLAPSSKSTSGGTAALGCLVKDYFPEPVTVSWNSGALTSGVHTFPAVLQSSGLYSLSSVVTVPSSSLGTQTYICNVNHKPSNTKVDKKVEPKSCDKTHTCPPCPAPEAAGGPSVFLFPPKPKDTLMISRTPEVTCVVVDVSHEDPEVKFNWYVDGVEVHNAKTKPREEQYNSTYRVVSVLTVLHQDWLNGKEYKCKVSNKALGAPIEKTISKAKGQPREPQVYTLPPSRDELTKNQVSLTCLVKGFYPSDIAVEWESNGQPENNYKTTPPVLDSDGSFFLYSKLTVDKSRWQQGNVFSCSVMHEALHNHYTQKSLSLSPG

SEQ ID NO: 72 - protein, 326 aa, synthetic construct
  REGION 1..326: note = human heavy chain constant region derived from IgG4
ASTKGPSVFPLAPCSRSTSESTAALGCLVKDYFPEPVTVSWNSGALTSGVHTFPAVLQSSGLYSLSSVVTVPSSSLGTKTYTCNVDHKPSNTKVDKRVESKYGPPCPSCPAPEFLGGPSVFLFPPKPKDTLMISRTPEVTCVVVDVSQEDPEVQFNWYVDGVEVHNAKTKPREEQFNSTYRVVSVLTVLHQDWLNGKEYKCKVSNKGLPSSIEKTISKAKGQPREPQVYTLPPSQEEMTKNQVSLTCLVKGFYPSDIAVEWESNGQPENNYKTTPPVLDSDGSFFLYSRLTVDKSRWQEGNVFSCSVMHEALHNHYTQKSLSLSLG

SEQ ID NO: 73 - protein, 497 aa, Homo sapiens
VPVVWAQEGAPAQLPCSPTIPLQDLSLLRRAGVTWQHQPDSGPPAAAPGHPLAPGPHPAAPSSWGPRPRRYTVLSVGPGGLRSGRLPLQPRVQLDERGRQRGDFSLWLRPARRADAGEYRAAVHLRDRALSCRLRLRLGQASMTASPPGSLRASDWVILNCSFSRPDRPASVHWFRNRGQGRVPVRESPHHHLAESFLFLPQVSPMDSGPWGCILTYRDGFNVSIMYNLTVLGLEPPTPLTVYAGAGSRVGLPCRLPAGVGTRSFLTAKWTPPGGGPDLLVTGDNGDFTLRLEDVSQAQAGTYTCHIHLQEQQLNATVTLAIITVTPKSFGSPGSLGKLLCEVTPVSGQERFVWSSLDTPSQRSFSGPWLEAQEAQLLSQPWQCQLYQGERLLGAAVYFTELSSPGAQRSGRAPGALPAGHLLLFLILGVLSLLLLVTGAFGFHLWRRQWRPRRFSALEQGIHPPQAQSKIEELEQEPEPEPEPEPEPEPEPEPEQL

SEQ ID NO: 74 - protein, 422 aa, Homo sapiens
VPVVWAQEGAPAQLPCSPTIPLQDLSLLRRAGVTWQHQPDSGPPAAAPGHPLAPGPHPAAPSSWGPRPRRYTVLSVGPGGLRSGRLPLQPRVQLDERGRQRGDFSLWLRPARRADAGEYRAAVHLRDRALSCRLRLRLGQASMTASPPGSLRASDWVILNCSFSRPDRPASVHWFRNRGQGRVPVRESPHHHLAESFLFLPQVSPMDSGPWGCILTYRDGFNVSIMYNLTVLGLEPPTPLTVYAGAGSRVGLPCRLPAGVGTRSFLTAKWTPPGGGPDLLVTGDNGDFTLRLEDVSQAQAGTYTCHIHLQEQQLNATVTLAIITVTPKSFGSPGSLGKLLCEVTPVSGQERFVWSSLDTPSQRSFSGPWLEAQEAQLLSQPWQCQLYQGERLLGAAVYFTELSSPGAQRSGRAPGALPAGHL

SEQ ID NO: 75 - protein, 6 aa, Homo sapiens
KIEELE

SEQ ID NO: 76 - DNA, 37 bp, synthetic construct
  misc_feature 1..37: note = primer rbHC.up
  source 1..37: mol_type = other DNA
aagcttgccaccatggagactgggctgcgctggcttc

SEQ ID NO: 77 - DNA, 21 bp, synthetic construct
  misc_feature 1..21: note = primer rbHCf.do
  source 1..21: mol_type = other DNA
ccattggtgagggtgcccgag

SEQ ID NO: 78 - DNA, 20 bp, synthetic construct
  misc_feature 1..20: note = primer BcPCR_FHLC_leader.fw
  source 1..20: mol_type = other DNA
atggacatgagggtccccgc

SEQ ID NO: 79 - DNA, 24 bp, synthetic construct
  misc_feature 1..24: note = primer BcPCR_huCkappa.rev
  source 1..24: mol_type = other DNA
gatttcaactgctcatcagatggc

SEQ ID NO: 80 - protein, 8 aa, synthetic construct
  REGION 1..8: note = heavy chain HVR-H1, PD1-0098
GYSITSDY

SEQ ID NO: 81 - skipped

SEQ ID NO: 82 - protein, 9 aa, synthetic construct
  REGION 1..9: note = heavy chain HVR-H3, PD1-0098
HGSAPWYFD

SEQ ID NO: 83 - protein, 12 aa, synthetic construct
  REGION 1..12: note = light chain HVR-L1, PD1-0098
SQNIVHSDGNTY

SEQ ID NO: 84 - skipped

SEQ ID NO: 85 - protein, 6 aa, synthetic construct
  REGION 1..6: note = light chain HVR-L3, PD1-0098
GSHFPL

SEQ ID NO: 86 - protein, 120 aa, synthetic construct
  REGION 1..120: note = heavy chain variable domain VH, PD1-0098
DVQLQESGPGLVKPSQSLSLTCTVTGYSITSDYAWNWIRQFPGDKLEWLGYITYSGFTNYNPSLKSRISISRDTSKNQFFLQLNSVATEDTATYYCARWHGSAPWYFDYWGRGTTLTVSS

SEQ ID NO: 87 - protein, 112 aa, synthetic construct
  REGION 1..112: note = light chain variable domain VL, PD1-0098
DVLMTQTPLSLPVSLGDQASISCRSSQNIVHSDGNTYLEWYLQKPGQSPNLLIYKVSRRFSGVPDRFSGSGSGTDFTLKISRVEAEDLGVYYCFQGSHFPLTFGAGTKLELK

SEQ ID NO: 88 - protein, 7 aa, synthetic construct
  REGION 1..7: note = heavy chain HVR-H1, PD1-0069
GYTFTDY

SEQ ID NO: 89 - skipped

SEQ ID NO: 90 - protein, 7 aa, synthetic construct
  REGION 1..7: note = heavy chain HVR-H3, PD1-0069
GITTGFA

SEQ ID NO: 91 - protein, 11 aa, synthetic construct
  REGION 1..11: note = light chain HVR-L1, PD1-0069
SKGVSTSSYSF

SEQ ID NO: 92 - skipped

SEQ ID NO: 93 - protein, 6 aa, synthetic construct
  REGION 1..6: note = light chain HVR-L3, PD1-0069
SREFPW

SEQ ID NO: 94 - protein, 118 aa, synthetic construct
  REGION 1..118: note = heavy chain variable domain VH, PD1-0069
QVQLQQSGPELVRPGVSVKISCKGSGYTFTDYAMHWVKQSHARTLEWIGVISTYSGDTNYNQKFKDKATMTVDKSSSTAYLELARMTSEDSAIYYCARLGITTGFAYWGQGTLVTVSA

SEQ ID NO: 95 - protein, 111 aa, synthetic construct
  REGION 1..111: note = light chain variable domain VL, PD1-0069
DIVLTQSPASLAVSLGQRATISCRASKGVSTSSYSFMHWYQQKPRQPPKLLIKYASYLESGVPARFSGSGSGTDFTLNIHPVEEEDAATYYCHHSREFPWTFGGGTKLEIK

SEQ ID NO: 96 - protein, 443 aa, synthetic construct
  REGION 1..443: note = heavy chain 1 of 1+1 PD1/LAG3 0799
DIVMTQSPDSLAVSLGERATINCKASESVDTSDNSFIHWYQQKPGQSPKLLIYRSSTLESGVPDRFSGSGSGTDFTLTISSLQAEDVAVYYCQQNYDVPWTFGQGTKVEIKSSASTKGPSVFPLAPSSKSTSGGTAALGCLVKDYFPEPVTVSWNSGALTSGVHTFPAVLQSSGLYSLSSVVTVPSSSLGTQTYICNVNHKPSNTKVDKKVEPKSCDKTHTCPPCPAPEAAGGPSVFLFPPKPKDTLMISRTPEVTCVVVDVSHEDPEVKFNWYVDGVEVHNAKTKPREEQYNSTYRVVSVLTVLHQDWLNGKEYKCKVSNKALGAPIEKTISKAKGQPREPQVYTLPPCRDELTKNQVSLWCLVKGFYPSDIAVEWESNGQPENNYKTTPPVLDSDGSFFLYSKLTVDKSRWQQGNVFSCSVMHEALHNHYTQKSLSLSPGK

SEQ ID NO: 97 - protein, 452 aa, synthetic construct
  REGION 1..452: note = heavy chain 2 of 1+1 PD1/LAG3 0799
EVQLVESGGGLVQPGGSLRLACAASGFTFSDYAMSWVRQAPGKGLEWVSGIDNSGYYTYYTDSVKGRFTISRDDVKNTLYLQMNSLRAEDTAVYLCTKTHSGLIVNDAFDIWGQGTMVTVSSASTKGPSVFPLAPSSKSTSGGTAALGCLVEDYFPEPVTVSWNSGALTSGVHTFPAVLQSSGLYSLSSVVTVPSSSLGTQTYICNVNHKPSNTKVDEKVEPKSCDKTHTCPPCPAPEAAGGPSVFLFPPKPKDTLMISRTPEVTCVVVDVSHEDPEVKFNWYVDGVEVHNAKTKPREEQYNSTYRVVSVLTVLHQDWLNGKEYKCKVSNKALGAPIEKTISKAKGQPREPQVCTLPPSRDELTKNQVSLSCAVKGFYPSDIAVEWESNGQPENNYKTTPPVLDSDGSFFLVSKLTVDKSRWQQGNVFSCSVMHEALHNHYTQKSLSLSPGK

SEQ ID NO: 98 - protein, 227 aa, synthetic construct
  REGION 1..227: note = light chain 1 of 1+1 PD1/LAG3 0799
EVQLLESGGGLVQPGGSLRLSCAASGFSFSSYTMSWVRQAPGKGLEWVATISGGGRDIYYPDSVKGRFTISRDNSKNTLYLQMNSLRAEDTAVYYCVLLTGRVYFALDSWGQGTLVTVSSASVAAPSVFIFPPSDEQLKSGTASVVCLLNNFYPREAKVQWKVDNALQSGNSQESVTEQDSKDSTYSLSSTLTLSKADYEKHKVYACEVTHQGLSSPVTKSFNRGEC

SEQ ID NO: 99 - protein, 214 aa, synthetic construct
  REGION 1..214: note = light chain 2 of 1+1 PD1/LAG3 0799
DIQLTQSPSSLSASVGDRVTITCRASQSISSYLNWYQQKPGKAPKLLIYDASSLESGVPSRFSGSGSGTDATLTISSLQPEDFATYYCQQSYSTPLTFGGGTKVEIKRTVAAPSVFIFPPSDRKLKSGTASVVCLLNNFYPREAKVQWKVDNALQSGNSQESVTEQDSKDSTYSLSSTLTLSKADYEKHKVYACEVTHQGLSSPVTKSFNRGEC

SEQ ID NO: 100 - protein, 451 aa, synthetic construct
  REGION 1..451: note = heavy chain 2 of 1+1 PD1/LAG3 0927
EVQLLESGGGLVQPGGSLRLSCAASGFIFDDYTMNWVRQAPGKGLEWVAVISWDGGGTYYTDSVKGRFTISRDDFKNTLYLQMNSLRAEDTAVYYCAKGLTDTTLYGSDYWGQGTLVTVSSASTKGPSVFPLAPSSKSTSGGTAALGCLVEDYFPEPVTVSWNSGALTSGVHTFPAVLQSSGLYSLSSVVTVPSSSLGTQTYICNVNHKPSNTKVDEKVEPKSCDKTHTCPPCPAPEAAGGPSVFLFPPKPKDTLMISRTPEVTCVVVDVSHEDPEVKFNWYVDGVEVHNAKTKPREEQYNSTYRVVSVLTVLHQDWLNGKEYKCKVSNKALGAPIEKTISKAKGQPREPQVCTLPPSRDELTKNQVSLSCAVKGFYPSDIAVEWESNGQPENNYKTTPPVLDSDGSFFLVSKLTVDKSRWQQGNVFSCSVMHEALHNHYTQKSLSLSPGK

SEQ ID NO: 101 - protein, 214 aa, synthetic construct
  REGION 1..214: note = light chain 2 of 1+1 PD1/LAG3 0927
DIQMTQSPSSLSASVGDRVTITCRASQSISSYLNWYQQKPGKAPKLLIYAASTLQSGVPSRFSGSGSGTDFTLTISSLQPEDFATYYCQQTYSSPLTFGGGTKVEIKRTVAAPSVFIFPPSDRKLKSGTASVVCLLNNFYPREAKVQWKVDNALQSGNSQESVTEQDSKDSTYSLSSTLTLSKADYEKHKVYACEVTHQGLSSPVTKSFNRGEC

SEQ ID NO: 102 - protein, 443 aa, synthetic construct
  REGION 1..443: note = heavy chain 1 of 1+1 PD1/LAG3 0222
DIVLTQSPASLAVSLGQRATISCRASKGVSTSSYSFMHWYQQKPRQPPKLLIKYASYLESGVPARFSGSGSGTDFTLNIHPVEEEDAATYYCHHSREFPWTFGGGTKLEIKSSASTKGPSVFPLAPSSKSTSGGTAALGCLVKDYFPEPVTVSWNSGALTSGVHTFPAVLQSSGLYSLSSVVTVPSSSLGTQTYICNVNHKPSNTKVDKKVEPKSCDKTHTCPPCPAPEAAGGPSVFLFPPKPKDTLMISRTPEVTCVVVDVSHEDPEVKFNWYVDGVEVHNAKTKPREEQYNSTYRVVSVLTVLHQDWLNGKEYKCKVSNKALGAPIEKTISKAKGQPREPQVYTLPPCRDELTKNQVSLWCLVKGFYPSDIAVEWESNGQPENNYKTTPPVLDSDGSFFLYSKLTVDKSRWQQGNVFSCSVMHEALHNHYTQKSLSLSPGK

SEQ ID NO: 103 - protein, 450 aa, synthetic construct
  REGION 1..450: note = heavy chain 2 of 1+1 PD1/LAG3 0222
QVQLQQWGAGLLKPSETLSLTCAVYGGSFSDYYWNWIRQPPGKGLEWIGEINHNGNTNSNPSLKSRVTLSLDTSKNQFSLKLRSVTAADTAVYYCAFGYSDYEYNWFDPWGQGTLVTVSSASTKGPSVFPLAPSSKSTSGGTAALGCLVEDYFPEPVTVSWNSGALTSGVHTFPAVLQSSGLYSLSSVVTVPSSSLGTQTYICNVNHKPSNTKVDEKVEPKSCDKTHTCPPCPAPEAAGGPSVFLFPPKPKDTLMISRTPEVTCVVVDVSHEDPEVKFNWYVDGVEVHNAKTKPREEQYNSTYRVVSVLTVLHQDWLNGKEYKCKVSNKALGAPIEKTISKAKGQPREPQVCTLPPSRDELTKNQVSLSCAVKGFYPSDIAVEWESNGQPENNYKTTPPVLDSDGSFFLVSKLTVDKSRWQQGNVFSCSVMHEALHNHYTQKSLSLSPGK

SEQ ID NO: 104 - protein, 225 aa, synthetic construct
  REGION 1..225: note = light chain 1 of 1+1 PD1/LAG3 0222
QVQLQQSGPELVRPGVSVKISCKGSGYTFTDYAMHWVKQSHARTLEWIGVISTYSGDTNYNQKFKDKATMTVDKSSSTAYLELARMTSEDSAIYYCARLGITTGFAYWGQGTLVTVSAASVAAPSVFIFPPSDEQLKSGTASVVCLLNNFYPREAKVQWKVDNALQSGNSQESVTEQDSKDSTYSLSSTLTLSKADYEKHKVYACEVTHQGLSSPVTKSFNRGEC

SEQ ID NO: 105 - protein, 214 aa, synthetic construct
  REGION 1..214: note = light chain 2 of 1+1 PD1/LAG3 0222
EIVLTQSPATLSLSPGERATLSCRASQSISSYLAWYQQKPGQAPRLLIYDASNRATGIPARFSGSGSGTDFTLTISSLEPEDFAVYYCQQRSNWPLTFGQGTNLEIKRTVAAPSVFIFPPSDRKLKSGTASVVCLLNNFYPREAKVQWKVDNALQSGNSQESVTEQDSKDSTYSLSSTLTLSKADYEKHKVYACEVTHQGLSSPVTKSFNRGEC

SEQ ID NO: 106 - protein, 444 aa, synthetic construct
  REGION 1..444: note = heavy chain 1 of 1+1 PD1/LAG3 0224
DVLMTQTPLSLPVSLGDQASISCRSSQNIVHSDGNTYLEWYLQKPGQSPNLLIYKVSRRFSGVPDRFSGSGSGTDFTLKISRVEAEDLGVYYCFQGSHFPLTFGAGTKLELKSSASTKGPSVFPLAPSSKSTSGGTAALGCLVKDYFPEPVTVSWNSGALTSGVHTFPAVLQSSGLYSLSSVVTVPSSSLGTQTYICNVNHKPSNTKVDKKVEPKSCDKTHTCPPCPAPEAAGGPSVFLFPPKPKDTLMISRTPEVTCVVVDVSHEDPEVKFNWYVDGVEVHNAKTKPREEQYNSTYRVVSVLTVLHQDWLNGKEYKCKVSNKALGAPIEKTISKAKGQPREPQVYTLPPCRDELTKNQVSLWCLVKGFYPSDIAVEWESNGQPENNYKTTPPVLDSDGSFFLYSKLTVDKSRWQQGNVFSCSVMHEALHNHYTQKSLSLSPGK

SEQ ID NO: 107 - protein, 227 aa, synthetic construct
  REGION 1..227: note = light chain 1 of 1+1 PD1/LAG3 0224
DVQLQESGPGLVKPSQSLSLTCTVTGYSITSDYAWNWIRQFPGDKLEWLGYITYSGFTNYNPSLKSRISISRDTSKNQFFLQLNSVATEDTATYYCARWHGSAPWYFDYWGRGTTLTVSSASVAAPSVFIFPPSDEQLKSGTASVVCLLNNFYPREAKVQWKVDNALQSGNSQESVTEQDSKDSTYSLSSTLTLSKADYEKHKVYACEVTHQGLSSPVTKSFNRGEC

SEQ ID NO: 108 - protein, 443 aa, synthetic construct
  REGION 1..443: note = aLAG3(0156) heavy chain (MDX25F7)
QVQLQQWGAGLLKPSETLSLTCAVYGGSFSDYYWNWIRQPPGKGLEWIGEINHNGNTNSNPSLKSRVTLSLDTSKNQFSLKLRSVTAADTAVYYCAFGYSDYEYNWFDPWGQGTLVTVSSGQPKAPSVFPLAPCCGDTPSSTVTLGCLVKGYLPEPVTVTWNSGTLTNGVRTFPSVRQSSGLYSLSSVVSVTSSSQPVTCNVAHPATNTKVDKTVAPSTCSKPTCPPPELLGGPSVFIFPPKPKDTLMISRTPEVTCVVVDVSQDDPEVQFTWYINNEQVRTARPPLREQQFNSTIRVVSTLPIAHQDWLRGKEFKCKVHNKALPAPIEKTISKARGQPLEPKVYTMGPPREELSSRSVSLTCMINGFYPSDISVEWEKNGKAEDNYKTTPAVLDSDGSYFLYNKLSVPTSEWQRGDVFTCSVMHEALHNHYTQKSISRSPGK

SEQ ID NO: 109 - protein, 214 aa, synthetic construct
  REGION 1..214: note = aLAG3(0156) light chain (MDX25F7)
EIVLTQSPATLSLSPGERATLSCRASQSISSYLAWYQQKPGQAPRLLIYDASNRATGIPARFSGSGSGTDFTLTISSLEPEDFAVYYCQQRSNWPLTFGQGTNLEIKRTVAAPSVFIFPPSDEQLKSGTASVVCLLNNFYPREAKVQWKVDNALQSGNSQESVTEQDSKDSTYSLSSTLTLSKADYEKHKVYACEVTHQGLSSPVTKSFNRGEC

SEQ ID NO: 110 - protein, 444 aa, synthetic construct
  REGION 1..444: note = aLAG3(0414) heavy chain
EVQLLESGGGLVQPGGSLRLSCAASGFIFDDYTMNWVRQAPGKGLEWVAVISWDGGGTYYTDSVKGRFTISRDDFKNTLYLQMNSLRAEDTAVYYCAKGLTDTTLYGSDYWGQGTLVTVSSGQPKAPSVFPLAPCCGDTPSSTVTLGCLVKGYLPEPVTVTWNSGTLTNGVRTFPSVRQSSGLYSLSSVVSVTSSSQPVTCNVAHPATNTKVDKTVAPSTCSKPTCPPPELLGGPSVFIFPPKPKDTLMISRTPEVTCVVVDVSQDDPEVQFTWYINNEQVRTARPPLREQQFNSTIRVVSTLPIAHQDWLRGKEFKCKVHNKALPAPIEKTISKARGQPLEPKVYTMGPPREELSSRSVSLTCMINGFYPSDISVEWEKNGKAEDNYKTTPAVLDSDGSYFLYNKLSVPTSEWQRGDVFTCSVMHEALHNHYTQKSISRSPGK

SEQ ID NO: 111 - protein, 214 aa, synthetic construct
  REGION 1..214: note = aLAG3(0414) light chain
DIQMTQSPSSLSASVGDRVTITCRASQSISSYLNWYQQKPGKAPKLLIYAASTLQSGVPSRFSGSGSGTDFTLTISSLQPEDFATYYCQQTYSSPLTFGGGTKVEIKGTVAAPSVFIFPPSDEQLKSGTASVVCLLNNFYPREAKVQWKVDNALQSGNSQESVTEQDSKDSTYSLSSTLTLSKADYEKHKVYACEVTHQGLSSPVTKSFNRGEC

SEQ ID NO: 112 - protein, 445 aa, synthetic construct
  REGION 1..445: note = aLAG3(0416) heavy chain
EVQLVESGGGLVQPGGSLRLACAASGFTFSDYAMSWVRQAPGKGLEWVSGIDNSGYYTYYTDSVKGRFTISRDDVKNTLYLQMNSLRAEDTAVYLCTKTHSGLIVNDAFDIWGQGTMVTVSSGQPKAPSVFPLAPCCGDTPSSTVTLGCLVKGYLPEPVTVTWNSGTLTNGVRTFPSVRQSSGLYSLSSVVSVTSSSQPVTCNVAHPATNTKVDKTVAPSTCSKPTCPPPELLGGPSVFIFPPKPKDTLMISRTPEVTCVVVDVSQDDPEVQFTWYINNEQVRTARPPLREQQFNSTIRVVSTLPIAHQDWLRGKEFKCKVHNKALPAPIEKTISKARGQPLEPKVYTMGPPREELSSRSVSLTCMINGFYPSDISVEWEKNGKAEDNYKTTPAVLDSDGSYFLYNKLSVPTSEWQRGDVFTCSVMHEALHNHYTQKSISRSPGK

SEQ ID NO: 113 - protein, 214 aa, synthetic construct
  REGION 1..214: note = aLAG3(0416) light chain
DIQLTQSPSSLSASVGDRVTITCRASQSISSYLNWYQQKPGKAPKLLIYDASSLESGVPSRFSGSGSGTDATLTISSLQPEDFATYYCQQSYSTPLTFGGGTKVEIKGTVAAPSVFIFPPSDEQLKSGTASVVCLLNNFYPREAKVQWKVDNALQSGNSQESVTEQDSKDSTYSLSSTLTLSKADYEKHKVYACEVTHQGLSSPVTKSFNRGEC

SEQ ID NO: 114 - protein, 695 aa, synthetic construct
  REGION 1..695: note = heavy chain of 2+2 PD1/LAG3 8970
EVQLLESGGGLVQPGGSLRLSCAASGFIFDDYTMNWVRQAPGKGLEWVAVISWDGGGTYYTDSVKGRFTISRDDFKNTLYLQMNSLRAEDTAVYYCAKGLTDTTLYGSDYWGQGTLVTVSSASTKGPSVFPLAPSSKSTSGGTAALGCLVEDYFPEPVTVSWNSGALTSGVHTFPAVLQSSGLYSLSSVVTVPSSSLGTQTYICNVNHKPSNTKVDEKVEPKSCDKTHTCPPCPAPEAAGGPSVFLFPPKPKDTLMISRTPEVTCVVVDVSHEDPEVKFNWYVDGVEVHNAKTKPREEQYNSTYRVVSVLTVLHQDWLNGKEYKCKVSNKALGAPIEKTISKAKGQPREPQVYTLPPSRDELTKNQVSLTCLVKGFYPSDIAVEWESNGQPENNYKTTPPVLDSDGSFFLYSKLTVDKSRWQQGNVFSCSVMHEALHNHYTQKSLSLSPGGGSGGGGSGGGGSGGGGSEVQLLESGGGLVQPGGSLRLSCAASGFSFSSYTMSWVRQAPGKGLEWVATISGGGRDIYYPDSVKGRFTISRDNSKNTLYLQMNSLRAEDTAVYYCVLLTGRVYFALDSWGQGTLVTVSSASVAAPSVFIFPPSDEQLKSGTASVVCLLNNFYPREAKVQWKVDNALQSGNSQESVTEQDSKDSTYSLSSTLTLSKADYEKHKVYACEVTHQGLSSPVTKSFNRGEC

SEQ ID NO: 115 - protein, 216 aa, synthetic construct
  REGION 1..216: note = light chain 1 of 2+2 PD1/LAG3 8970
DIVMTQSPDSLAVSLGERATINCKASESVDTSDNSFIHWYQQKPGQSPKLLIYRSSTLESGVPDRFSGSGSGTDFTLTISSLQAEDVAVYYCQQNYDVPWTFGQGTKVEIKSSASTKGPSVFPLAPSSKSTSGGTAALGCLVKDYFPEPVTVSWNSGALTSGVHTFPAVLQSSGLYSLSSVVTVPSSSLGTQTYICNVNHKPSNTKVDKKVEPKSC

SEQ ID NO: 116 - protein, 696 aa, synthetic construct
  REGION 1..696: note = heavy chain of 2+2 PD1/LAG3 8984
EVQLVESGGGLVQPGGSLRLACAASGFTFSDYAMSWVRQAPGKGLEWVSGIDNSGYYTYYTDSVKGRFTISRDDVKNTLYLQMNSLRAEDTAVYLCTKTHSGLIVNDAFDIWGQGTMVTVSSASTKGPSVFPLAPSSKSTSGGTAALGCLVEDYFPEPVTVSWNSGALTSGVHTFPAVLQSSGLYSLSSVVTVPSSSLGTQTYICNVNHKPSNTKVDEKVEPKSCDKTHTCPPCPAPEAAGGPSVFLFPPKPKDTLMISRTPEVTCVVVDVSHEDPEVKFNWYVDGVEVHNAKTKPREEQYNSTYRVVSVLTVLHQDWLNGKEYKCKVSNKALGAPIEKTISKAKGQPREPQVYTLPPSRDELTKNQVSLTCLVKGFYPSDIAVEWESNGQPENNYKTTPPVLDSDGSFFLYSKLTVDKSRWQQGNVFSCSVMHEALHNHYTQKSLSLSPGGGSGGGGSGGGGSGGGGSEVQLLESGGGLVQPGGSLRLSCAASGFSFSSYTMSWVRQAPGKGLEWVATISGGGRDIYYPDSVKGRFTISRDNSKNTLYLQMNSLRAEDTAVYYCVLLTGRVYFALDSWGQGTLVTVSSASVAAPSVFIFPPSDEQLKSGTASVVCLLNNFYPREAKVQWKVDNALQSGNSQESVTEQDSKDSTYSLSSTLTLSKADYEKHKVYACEVTHQGLSSPVTKSFNRGEC

SEQ ID NO: 117 - protein, 694 aa, synthetic construct
  REGION 1..694: note = heavy chain of 2+2 PD1/LAG3 9010
QVQLQQWGAGLLKPSETLSLTCAVYGGSFSDYYWNWIRQPPGKGLEWIGEINHNGNTNSNPSLKSRVTLSLDTSKNQFSLKLRSVTAADTAVYYCAFGYSDYEYNWFDPWGQGTLVTVSSASTKGPSVFPLAPSSKSTSGGTAALGCLVEDYFPEPVTVSWNSGALTSGVHTFPAVLQSSGLYSLSSVVTVPSSSLGTQTYICNVNHKPSNTKVDEKVEPKSCDKTHTCPPCPAPEAAGGPSVFLFPPKPKDTLMISRTPEVTCVVVDVSHEDPEVKFNWYVDGVEVHNAKTKPREEQYNSTYRVVSVLTVLHQDWLNGKEYKCKVSNKALGAPIEKTISKAKGQPREPQVYTLPPSRDELTKNQVSLTCLVKGFYPSDIAVEWESNGQPENNYKTTPPVLDSDGSFFLYSKLTVDKSRWQQGNVFSCSVMHEALHNHYTQKSLSLSPGGGSGGGGSGGGGSGGGGSEVQLLESGGGLVQPGGSLRLSCAASGFSFSSYTMSWVRQAPGKGLEWVATISGGGRDIYYPDSVKGRFTISRDNSKNTLYLQMNSLRAEDTAVYYCVLLTGRVYFALDSWGQGTLVTVSSASVAAPSVFIFPPSDEQLKSGTASVVCLLNNFYPREAKVQWKVDNALQSGNSQESVTEQDSKDSTYSLSSTLTLSKADYEKHKVYACEVTHQGLSSPVTKSFNRGEC

SEQ ID NO: 118 - protein, 695 aa, synthetic construct
  REGION 1..695: note = heavy chain 1of 2+1 PD1/LAG3 8310
EVQLLESGGGLVQPGGSLRLSCAASGFIFDDYTMNWVRQAPGKGLEWVAVISWDGGGTYYTDSVKGRFTISRDDFKNTLYLQMNSLRAEDTAVYYCAKGLTDTTLYGSDYWGQGTLVTVSSASTKGPSVFPLAPSSKSTSGGTAALGCLVEDYFPEPVTVSWNSGALTSGVHTFPAVLQSSGLYSLSSVVTVPSSSLGTQTYICNVNHKPSNTKVDEKVEPKSCDKTHTCPPCPAPEAAGGPSVFLFPPKPKDTLMISRTPEVTCVVVDVSHEDPEVKFNWYVDGVEVHNAKTKPREEQYNSTYRVVSVLTVLHQDWLNGKEYKCKVSNKALGAPIEKTISKAKGQPREPQVYTLPPCRDELTKNQVSLWCLVKGFYPSDIAVEWESNGQPENNYKTTPPVLDSDGSFFLYSKLTVDKSRWQQGNVFSCSVMHEALHNHYTQKSLSLSPGGGSGGGGSGGGGSGGGGSEVQLLESGGGLVQPGGSLRLSCAASGFSFSSYTMSWVRQAPGKGLEWVATISGGGRDIYYPDSVKGRFTISRDNSKNTLYLQMNSLRAEDTAVYYCVLLTGRVYFALDSWGQGTLVTVSSASVAAPSVFIFPPSDEQLKSGTASVVCLLNNFYPREAKVQWKVDNALQSGNSQESVTEQDSKDSTYSLSSTLTLSKADYEKHKVYACEVTHQGLSSPVTKSFNRGEC

SEQ ID NO: 119 - protein, 451 aa, synthetic construct; identical to SEQ ID NO: 100
  REGION 1..451: note = heavy chain 2 of 2+1 PD1/LAG3 8310

SEQ ID NO: 120 - protein, 696 aa, synthetic construct
  REGION 1..696: note = heavy chain 1of 2+1 PD1/LAG3 8311
EVQLVESGGGLVQPGGSLRLACAASGFTFSDYAMSWVRQAPGKGLEWVSGIDNSGYYTYYTDSVKGRFTISRDDVKNTLYLQMNSLRAEDTAVYLCTKTHSGLIVNDAFDIWGQGTMVTVSSASTKGPSVFPLAPSSKSTSGGTAALGCLVEDYFPEPVTVSWNSGALTSGVHTFPAVLQSSGLYSLSSVVTVPSSSLGTQTYICNVNHKPSNTKVDEKVEPKSCDKTHTCPPCPAPEAAGGPSVFLFPPKPKDTLMISRTPEVTCVVVDVSHEDPEVKFNWYVDGVEVHNAKTKPREEQYNSTYRVVSVLTVLHQDWLNGKEYKCKVSNKALGAPIEKTISKAKGQPREPQVYTLPPCRDELTKNQVSLWCLVKGFYPSDIAVEWESNGQPENNYKTTPPVLDSDGSFFLYSKLTVDKSRWQQGNVFSCSVMHEALHNHYTQKSLSLSPGGGSGGGGSGGGGSGGGGSEVQLLESGGGLVQPGGSLRLSCAASGFSFSSYTMSWVRQAPGKGLEWVATISGGGRDIYYPDSVKGRFTISRDNSKNTLYLQMNSLRAEDTAVYYCVLLTGRVYFALDSWGQGTLVTVSSASVAAPSVFIFPPSDEQLKSGTASVVCLLNNFYPREAKVQWKVDNALQSGNSQESVTEQDSKDSTYSLSSTLTLSKADYEKHKVYACEVTHQGLSSPVTKSFNRGEC

SEQ ID NO: 121 - protein, 452 aa, synthetic construct; identical to SEQ ID NO: 97
  REGION 1..452: note = heavy chain 2of 2+1 PD1/LAG3 8311

SEQ ID NO: 122 - protein, 694 aa, synthetic construct
  REGION 1..694: note = heavy chain 1of 2+1 PD1/LAG3 1252
QVQLQQWGAGLLKPSETLSLTCAVYGGSFSDYYWNWIRQPPGKGLEWIGEINHNGNTNSNPSLKSRVTLSLDTSKNQFSLKLRSVTAADTAVYYCAFGYSDYEYNWFDPWGQGTLVTVSSASTKGPSVFPLAPSSKSTSGGTAALGCLVEDYFPEPVTVSWNSGALTSGVHTFPAVLQSSGLYSLSSVVTVPSSSLGTQTYICNVNHKPSNTKVDEKVEPKSCDKTHTCPPCPAPEAAGGPSVFLFPPKPKDTLMISRTPEVTCVVVDVSHEDPEVKFNWYVDGVEVHNAKTKPREEQYNSTYRVVSVLTVLHQDWLNGKEYKCKVSNKALGAPIEKTISKAKGQPREPQVYTLPPCRDELTKNQVSLWCLVKGFYPSDIAVEWESNGQPENNYKTTPPVLDSDGSFFLYSKLTVDKSRWQQGNVFSCSVMHEALHNHYTQKSLSLSPGGGSGGGGSGGGGSGGGGSEVQLLESGGGLVQPGGSLRLSCAASGFSFSSYTMSWVRQAPGKGLEWVATISGGGRDIYYPDSVKGRFTISRDNSKNTLYLQMNSLRAEDTAVYYCVLLTGRVYFALDSWGQGTLVTVSSASVAAPSVFIFPPSDEQLKSGTASVVCLLNNFYPREAKVQWKVDNALQSGNSQESVTEQDSKDSTYSLSSTLTLSKADYEKHKVYACEVTHQGLSSPVTKSFNRGEC

SEQ ID NO: 123 - protein, 941 aa, synthetic construct
  REGION 1..941: note = heavy chain 1of 2+1 PD1/LAG3 8312
EVQLLESGGGLVQPGGSLRLSCAASGFIFDDYTMNWVRQAPGKGLEWVAVISWDGGGTYYTDSVKGRFTISRDDFKNTLYLQMNSLRAEDTAVYYCAKGLTDTTLYGSDYWGQGTLVTVSSASTKGPSVFPLAPSSKSTSGGTAALGCLVEDYFPEPVTVSWNSGALTSGVHTFPAVLQSSGLYSLSSVVTVPSSSLGTQTYICNVNHKPSNTKVDEKVEPKSCDKTHTCPPCPAPEAAGGPSVFLFPPKPKDTLMISRTPEVTCVVVDVSHEDPEVKFNWYVDGVEVHNAKTKPREEQYNSTYRVVSVLTVLHQDWLNGKEYKCKVSNKALGAPIEKTISKAKGQPREPQVYTLPPCRDELTKNQVSLWCLVKGFYPSDIAVEWESNGQPENNYKTTPPVLDSDGSFFLYSKLTVDKSRWQQGNVFSCSVMHEALHNHYTQKSLSLSPGGGGGSGGGGSGGGGSGGGGSDIVMTQSPDSLAVSLGERATINCKASESVDTSDNSFIHWYQQKPGQSPKLLIYRSSTLESGVPDRFSGSGSGTDFTLTISSLQAEDVAVYYCQQNYDVPWTFGQGTKVEIKRTVAAPSVFIFPPSDEQLKSGTASVVCLLNNFYPREAKVQWKVDNALQSGNSQESVTEQDSKDSTYSLSSTLTLSKADYEKHKVYACEVTHQGLSSPVTKSFNRGECGGGGSGGGGSGGGGSGGGGSGGGGSGGGGSEVQLLESGGGLVQPGGSLRLSCAASGFSFSSYTMSWVRQAPGKGLEWVATISGGGRDIYYPDSVKGRFTISRDNSKNTLYLQMNSLRAEDTAVYYCVLLTGRVYFALDSWGQGTLVTVSSASTKGPSVFPLAPSSKSTSGGTAALGCLVKDYFPEPVTVSWNSGALTSGVHTFPAVLQSSGLYSLSSVVTVPSSSLGTQTYICNVNHKPSNTKVDKKVEPKSC

SEQ ID NO: 124 - protein, 942 aa, synthetic construct
  REGION 1..942: note = heavy chain 1of 2+1 PD1/LAG3 8313
EVQLVESGGGLVQPGGSLRLACAASGFTFSDYAMSWVRQAPGKGLEWVSGIDNSGYYTYYTDSVKGRFTISRDDVKNTLYLQMNSLRAEDTAVYLCTKTHSGLIVNDAFDIWGQGTMVTVSSASTKGPSVFPLAPSSKSTSGGTAALGCLVEDYFPEPVTVSWNSGALTSGVHTFPAVLQSSGLYSLSSVVTVPSSSLGTQTYICNVNHKPSNTKVDEKVEPKSCDKTHTCPPCPAPEAAGGPSVFLFPPKPKDTLMISRTPEVTCVVVDVSHEDPEVKFNWYVDGVEVHNAKTKPREEQYNSTYRVVSVLTVLHQDWLNGKEYKCKVSNKALGAPIEKTISKAKGQPREPQVYTLPPCRDELTKNQVSLWCLVKGFYPSDIAVEWESNGQPENNYKTTPPVLDSDGSFFLYSKLTVDKSRWQQGNVFSCSVMHEALHNHYTQKSLSLSPGGGGGSGGGGSGGGGSGGGGSDIVMTQSPDSLAVSLGERATINCKASESVDTSDNSFIHWYQQKPGQSPKLLIYRSSTLESGVPDRFSGSGSGTDFTLTISSLQAEDVAVYYCQQNYDVPWTFGQGTKVEIKRTVAAPSVFIFPPSDEQLKSGTASVVCLLNNFYPREAKVQWKVDNALQSGNSQESVTEQDSKDSTYSLSSTLTLSKADYEKHKVYACEVTHQGLSSPVTKSFNRGECGGGGSGGGGSGGGGSGGGGSGGGGSGGGGSEVQLLESGGGLVQPGGSLRLSCAASGFSFSSYTMSWVRQAPGKGLEWVATISGGGRDIYYPDSVKGRFTISRDNSKNTLYLQMNSLRAEDTAVYYCVLLTGRVYFALDSWGQGTLVTVSSASTKGPSVFPLAPSSKSTSGGTAALGCLVKDYFPEPVTVSWNSGALTSGVHTFPAVLQSSGLYSLSSVVTVPSSSLGTQTYICNVNHKPSNTKVDKKVEPKSC

SEQ ID NO: 125 - protein, 940 aa, synthetic construct
  REGION 1..940: note = heavy chain 1of 2+1 PD1/LAG3 1088
QVQLQQWGAGLLKPSETLSLTCAVYGGSFSDYYWNWIRQPPGKGLEWIGEINHNGNTNSNPSLKSRVTLSLDTSKNQFSLKLRSVTAADTAVYYCAFGYSDYEYNWFDPWGQGTLVTVSSASTKGPSVFPLAPSSKSTSGGTAALGCLVEDYFPEPVTVSWNSGALTSGVHTFPAVLQSSGLYSLSSVVTVPSSSLGTQTYICNVNHKPSNTKVDEKVEPKSCDKTHTCPPCPAPEAAGGPSVFLFPPKPKDTLMISRTPEVTCVVVDVSHEDPEVKFNWYVDGVEVHNAKTKPREEQYNSTYRVVSVLTVLHQDWLNGKEYKCKVSNKALGAPIEKTISKAKGQPREPQVYTLPPCRDELTKNQVSLWCLVKGFYPSDIAVEWESNGQPENNYKTTPPVLDSDGSFFLYSKLTVDKSRWQQGNVFSCSVMHEALHNHYTQKSLSLSPGGGGGSGGGGSGGGGSGGGGSDIVMTQSPDSLAVSLGERATINCKASESVDTSDNSFIHWYQQKPGQSPKLLIYRSSTLESGVPDRFSGSGSGTDFTLTISSLQAEDVAVYYCQQNYDVPWTFGQGTKVEIKRTVAAPSVFIFPPSDEQLKSGTASVVCLLNNFYPREAKVQWKVDNALQSGNSQESVTEQDSKDSTYSLSSTLTLSKADYEKHKVYACEVTHQGLSSPVTKSFNRGECGGGGSGGGGSGGGGSGGGGSGGGGSGGGGSEVQLLESGGGLVQPGGSLRLSCAASGFSFSSYTMSWVRQAPGKGLEWVATISGGGRDIYYPDSVKGRFTISRDNSKNTLYLQMNSLRAEDTAVYYCVLLTGRVYFALDSWGQGTLVTVSSASTKGPSVFPLAPSSKSTSGGTAALGCLVKDYFPEPVTVSWNSGALTSGVHTFPAVLQSSGLYSLSSVVTVPSSSLGTQTYICNVNHKPSNTKVDKKVEPKSC

SEQ ID NO: 126 - protein, 589 aa, synthetic construct
  REGION 1..589: note = heavy chain 1of 2+1 PD1/LAG3 0918
QVQLQQWGAGLLKPSETLSLTCAVYGGSFSDYYWNWIRQPPGKGLEWIGEINHNGNTNSNPSLKSRVTLSLDTSKNQFSLKLRSVTAADTAVYYCAFGYSDYEYNWFDPWGQGTLVTVSSASTKGPSVFPLAPSSKSTSGGTAALGCLVKDYFPEPVTVSWNSGALTSGVHTFPAVLQSSGLYSLSSVVTVPSSSLGTQTYICNVNHKPSNTKVDKKVEPKSCDKTHTCPPCPAPEAAGGPSVFLFPPKPKDTLMISRTPEVTCVVVDVSHEDPEVKFNWYVDGVEVHNAKTKPREEQYNSTYRVVSVLTVLHQDWLNGKEYKCKVSNKALGAPIEKTISKAKGQPREPQVCTLPPSRDELTKNQVSLSCAVKGFYPSDIAVEWESNGQPENNYKTTPPVLDSDGSFFLVSKLTVDKSRWQQGNVFSCSVMHEALHNHYTQKSLSLSPGGGGGSGGGGSGGGGSGGGGSEVQLLESGGGLVQPGGSLRLSCAASGFSFSSYTMSWVRQAPGKGLEWVATISGGGRDIYYPDSVKGRFTISRDNSKNTLYLQMNSLRAEDTAVYYCVLLTGRVYFALDSWGQGTLVTVSS

SEQ ID NO: 127 - protein, 580 aa, synthetic construct
  REGION 1..580: note = heavy chain 2 of 2+1 PD1/LAG3 0918
QVQLQQWGAGLLKPSETLSLTCAVYGGSFSDYYWNWIRQPPGKGLEWIGEINHNGNTNSNPSLKSRVTLSLDTSKNQFSLKLRSVTAADTAVYYCAFGYSDYEYNWFDPWGQGTLVTVSSASTKGPSVFPLAPSSKSTSGGTAALGCLVKDYFPEPVTVSWNSGALTSGVHTFPAVLQSSGLYSLSSVVTVPSSSLGTQTYICNVNHKPSNTKVDKKVEPKSCDKTHTCPPCPAPEAAGGPSVFLFPPKPKDTLMISRTPEVTCVVVDVSHEDPEVKFNWYVDGVEVHNAKTKPREEQYNSTYRVVSVLTVLHQDWLNGKEYKCKVSNKALGAPIEKTISKAKGQPREPQVYTLPPCRDELTKNQVSLWCLVKGFYPSDIAVEWESNGQPENNYKTTPPVLDSDGSFFLYSKLTVDKSRWQQGNVFSCSVMHEALHNHYTQKSLSLSPGGGGGSGGGGSGGGGSGGGGSDIVMTQSPDSLAVSLGERATINCKASESVDTSDNSFIHWYQQKPGQSPKLLIYRSSTLESGVPDRFSGSGSGTDFTLTISSLQAEDVAVYYCQQNYDVPWTFGQGTKVEIK

SEQ ID NO: 128 - protein, 288 aa, Homo sapiens
MQIPQAPWPVVWAVLQLGWRPGWFLDSPDRPWNPPTFSPALLVVTEGDNATFTCSFSNTSESFVLNWYRMSPSNQTDKLAAFPEDRSQPGQDCRFRVTQLPNGRDFHMSVVRARRNDSGTYLCGAISLAPKAQIKESLRAELRVTERRAEVPTAHPSPSPRPAGQFQTLVVGVVGGLLGSLVLLVWVLAVICSRAARGTIGARRTGQPLKEDPSAVPVFSVDYGELDFQWREKTPEPPVPCVPEQTEYATIVFPSGMGTSSPARRGSADGPRSAQPLRPEDGHCSWPL

SEQ ID NO: 129 - protein, 5 aa, synthetic construct
  REGION 1..5: note = Peptide linker G4S
GGGGS

SEQ ID NO: 130 - protein, 10 aa, synthetic construct
  REGION 1..10: note = Peptide linker (G4S)2
GGGGSGGGGS

SEQ ID NO: 131 - protein, 10 aa, synthetic construct
  REGION 1..10: note = Peptide linker (SG4)2
SGGGGSGGGG

SEQ ID NO: 132 - protein, 14 aa, synthetic construct
  REGION 1..14: note = Peptide linker G4(SG4)2
GGGGSGGGGSGGGG

SEQ ID NO: 133 - protein, 10 aa, synthetic construct
  REGION 1..10: note = Peptide linker
GSPGSSSSGS

SEQ ID NO: 134 - protein, 15 aa, synthetic construct
  REGION 1..15: note = Peptide linker (G4S)3
GGGGSGGGGSGGGGS

SEQ ID NO: 135 - protein, 20 aa, synthetic construct
  REGION 1..20: note = Peptide linker (G4S)4
GGGGSGGGGSGGGGSGGGGS

SEQ ID NO: 136 - protein, 8 aa, synthetic construct
  REGION 1..8: note = Peptide linker
GSGSGSGS

SEQ ID NO: 137 - protein, 8 aa, synthetic construct
  REGION 1..8: note = Peptide linker
GSGSGNGS

SEQ ID NO: 138 - protein, 8 aa, synthetic construct
  REGION 1..8: note = Peptide linker
GGSGSGSG

SEQ ID NO: 139 - protein, 6 aa, synthetic construct
  REGION 1..6: note = Peptide linker
GGSGSG

SEQ ID NO: 140 - protein, 4 aa, synthetic construct
  REGION 1..4: note = Peptide linker
GGSG

SEQ ID NO: 141 - protein, 8 aa, synthetic construct
  REGION 1..8: note = Peptide linker
GGSGNGSG

SEQ ID NO: 142 - protein, 8 aa, synthetic construct
  REGION 1..8: note = Peptide linker
GGNGSGSG

SEQ ID NO: 143 - protein, 6 aa, synthetic construct
  REGION 1..6: note = Peptide linker
GGNGSG

SEQ ID NO: 144 - protein, 461 aa, synthetic construct
  REGION 1..461: note = heavy chain 2 of 1+1 PD1/LAG3 0725 (1+1 trans)
DKTHTCPPCPAPEAAGGPSVFLFPPKPKDTLMISRTPEVTCVVVDVSHEDPEVKFNWYVDGVEVHNAKTKPREEQYNSTYRVVSVLTVLHQDWLNGKEYKCKVSNKALGAPIEKTISKAKGQPREPQVCTLPPSRDELTKNQVSLSCAVKGFYPSDIAVEWESNGQPENNYKTTPPVLDSDGSFFLVSKLTVDKSRWQQGNVFSCSVMHEALHNHYTQKSLSLSPGKGGGGSGGGGSEVQLLESGGGLVQPGGSLRLSCAASGFIFDDYTMNWVRQAPGKGLEWVAVISWDGGGTYYTDSVKGRFTISRDDFKNTLYLQMNSLRAEDTAVYYCAKGLTDTTLYGSDYWGQGTLVTVSSASTKGPSVFPLAPSSKSTSGGTAALGCLVEDYFPEPVTVSWNSGALTSGVHTFPAVLQSSGLYSLSSVVTVPSSSLGTQTYICNVNHKPSNTKVDEKVEPKSC

SEQ ID NO: 145 - protein, 685 aa, synthetic construct
  REGION 1..685: note = heavy chain 2 of 2+1 PD1/LAG3 0750 (2+1 trans)
EVQLLESGGGLVQPGGSLRLSCAASGFIFDDYTMNWVRQAPGKGLEWVAVISWDGGGTYYTDSVKGRFTISRDDFKNTLYLQMNSLRAEDTAVYYCAKGLTDTTLYGSDYWGQGTLVTVSSASTKGPSVFPLAPSSKSTSGGTAALGCLVEDYFPEPVTVSWNSGALTSGVHTFPAVLQSSGLYSLSSVVTVPSSSLGTQTYICNVNHKPSNTKVDEKVEPKSCDKTHTCPPCPAPEAAGGPSVFLFPPKPKDTLMISRTPEVTCVVVDVSHEDPEVKFNWYVDGVEVHNAKTKPREEQYNSTYRVVSVLTVLHQDWLNGKEYKCKVSNKALGAPIEKTISKAKGQPREPQVCTLPPSRDELTKNQVSLSCAVKGFYPSDIAVEWESNGQPENNYKTTPPVLDSDGSFFLVSKLTVDKSRWQQGNVFSCSVMHEALHNHYTQKSLSLSPGKGGGGSGGGGSEVQLLESGGGLVQPGGSLRLSCAASGFIFDDYTMNWVRQAPGKGLEWVAVISWDGGGTYYTDSVKGRFTISRDDFKNTLYLQMNSLRAEDTAVYYCAKGLTDTTLYGSDYWGQGTLVTVSSASTKGPSVFPLAPSSKSTSGGTAALGCLVEDYFPEPVTVSWNSGALTSGVHTFPAVLQSSGLYSLSSVVTVPSSSLGTQTYICNVNHKPSNTKVDEKVEPKSC

SEQ ID NO: 146 - protein, 215 aa, synthetic construct
  REGION 1..215: note = Light chain CEA (CEA TCB)
DIQMTQSPSSLSASVGDRVTITCKASAAVGTYVAWYQQKPGKAPKLLIYSASYRKRGVPSRFSGSGSGTDFTLTISSLQPEDFATYYCHQYYTYPLFTFGQGTKLEIKRTVAAPSVFIFPPSDEQLKSGTASVVCLLNNFYPREAKVQWKVDNALQSGNSQESVTEQDSKDSTYSLSSTLTLSKADYEKHKVYACEVTHQGLSSPVTKSFNRGEC

SEQ ID NO: 147 - protein, 214 aa, synthetic construct
  REGION 1..214: note = Light chain CD3 (CEA TCB)
QAVVTQEPSLTVSPGGTVTLTCGSSTGAVTTSNYANWVQEKPGQAFRGLIGGTNKRAPGTPARFSGSLLGGKAALTLSGAQPEDEAEYYCALWYSNLWVFGGGTKLTVLSSASTKGPSVFPLAPSSKSTSGGTAALGCLVKDYFPEPVTVSWNSGALTSGVHTFPAVLQSSGLYSLSSVVTVPSSSLGTQTYICNVNHKPSNTKVDKKVEPKSC

SEQ ID NO: 148 - protein, 694 aa, synthetic construct
  REGION 1..694: note = CEA CD3 crossfab VHck fc knob P329GLALA (CEA TCB)
QVQLVQSGAEVKKPGASVKVSCKASGYTFTEFGMNWVRQAPGQGLEWMGWINTKTGEATYVEEFKGRVTFTTDTSTSTAYMELRSLRSDDTAVYYCARWDFAYYVEAMDYWGQGTTVTVSSASTKGPSVFPLAPSSKSTSGGTAALGCLVKDYFPEPVTVSWNSGALTSGVHTFPAVLQSSGLYSLSSVVTVPSSSLGTQTYICNVNHKPSNTKVDKKVEPKSCDGGGGSGGGGSEVQLLESGGGLVQPGGSLRLSCAASGFTFSTYAMNWVRQAPGKGLEWVSRIRSKYNNYATYYADSVKGRFTISRDDSKNTLYLQMNSLRAEDTAVYYCVRHGNFGNSYVSWFAYWGQGTLVTVSSASVAAPSVFIFPPSDEQLKSGTASVVCLLNNFYPREAKVQWKVDNALQSGNSQESVTEQDSKDSTYSLSSTLTLSKADYEKHKVYACEVTHQGLSSPVTKSFNRGECDKTHTCPPCPAPEAAGGPSVFLFPPKPKDTLMISRTPEVTCVVVDVSHEDPEVKFNWYVDGVEVHNAKTKPREEQYNSTYRVVSVLTVLHQDWLNGKEYKCKVSNKALGAPIEKTISKAKGQPREPQVYTLPPCRDELTKNQVSLWCLVKGFYPSDIAVEWESNGQPENNYKTTPPVLDSDGSFFLYSKLTVDKSRWQQGNVFSCSVMHEALHNHYTQKSLSLSPGK

SEQ ID NO: 149 - protein, 451 aa, synthetic construct
  REGION 1..451: note = CEA VHCH1 Fc hole P329GLALA (CEA TCB)
QVQLVQSGAEVKKPGASVKVSCKASGYTFTEFGMNWVRQAPGQGLEWMGWINTKTGEATYVEEFKGRVTFTTDTSTSTAYMELRSLRSDDTAVYYCARWDFAYYVEAMDYWGQGTTVTVSSASTKGPSVFPLAPSSKSTSGGTAALGCLVKDYFPEPVTVSWNSGALTSGVHTFPAVLQSSGLYSLSSVVTVPSSSLGTQTYICNVNHKPSNTKVDKKVEPKSCDKTHTCPPCPAPEAAGGPSVFLFPPKPKDTLMISRTPEVTCVVVDVSHEDPEVKFNWYVDGVEVHNAKTKPREEQYNSTYRVVSVLTVLHQDWLNGKEYKCKVSNKALGAPIEKTISKAKGQPREPQVCTLPPSRDELTKNQVSLSCAVKGFYPSDIAVEWESNGQPENNYKTTPPVLDSDGSFFLVSKLTVDKSRWQQGNVFSCSVMHEALHNHYTQKSLSLSPGK

SEQ ID NO: 150 - protein, 232 aa, synthetic construct
  REGION 1..232: note = CD3 VH-CL (CEACAM5 TCB)
EVQLLESGGGLVQPGGSLRLSCAASGFTFSTYAMNWVRQAPGKGLEWVSRIRSKYNNYATYYADSVKGRFTISRDDSKNTLYLQMNSLRAEDTAVYYCVRHGNFGNSYVSWFAYWGQGTLVTVSSASVAAPSVFIFPPSDEQLKSGTASVVCLLNNFYPREAKVQWKVDNALQSGNSQESVTEQDSKDSTYSLSSTLTLSKADYEKHKVYACEVTHQGLSSPVTKSFNRGEC

SEQ ID NO: 151 - protein, 449 aa, synthetic construct
  REGION 1..449: note = CEACAM5 VH-CH1(EE)-Fc (hole, P329G LALA)
QVQLVQSGAEVKKPGSSVKVSCKASGFNIKDTYMHWVRQAPGQGLEWMGRIDPANGNSKYVPKFQGRVTITADTSTSTAYMELSSLRSEDTAVYYCAPFGYYVSDYAMAYWGQGTLVTVSSASTKGPSVFPLAPSSKSTSGGTAALGCLVEDYFPEPVTVSWNSGALTSGVHTFPAVLQSSGLYSLSSVVTVPSSSLGTQTYICNVNHKPSNTKVDEKVEPKSCDKTHTCPPCPAPEAAGGPSVFLFPPKPKDTLMISRTPEVTCVVVDVSHEDPEVKFNWYVDGVEVHNAKTKPREEQYNSTYRVVSVLTVLHQDWLNGKEYKCKVSNKALGAPIEKTISKAKGQPREPQVCTLPPSRDELTKNQVSLSCAVKGFYPSDIAVEWESNGQPENNYKTTPPVLDSDGSFFLVSKLTVDKSRWQQGNVFSCSVMHEALHNHYTQKSLSLSP

SEQ ID NO: 152 - protein, 674 aa, synthetic construct
  REGION 1..674: note = CEACAM5 VH-CH1(EE)-CD3 VL-CH1-Fc (knob, P329G LALA)
QVQLVQSGAEVKKPGSSVKVSCKASGFNIKDTYMHWVRQAPGQGLEWMGRIDPANGNSKYVPKFQGRVTITADTSTSTAYMELSSLRSEDTAVYYCAPFGYYVSDYAMAYWGQGTLVTVSSASTKGPSVFPLAPSSKSTSGGTAALGCLVEDYFPEPVTVSWNSGALTSGVHTFPAVLQSSGLYSLSSVVTVPSSSLGTQTYICNVNHKPSNTKVDEKVEPKSCDGGGGSGGGGSQAVVTQEPSLTVSPGGTVTLTCGSSTGAVTTSNYANWVQEKPGQAFRGLIGGTNKRAPGTPARFSGSLLGGKAALTLSGAQPEDEAEYYCALWYSNLWVFGGGTKLTVLSSASTKGPSVFPLAPSSKSTSGGTAALGCLVKDYFPEPVTVSWNSGALTSGVHTFPAVLQSSGLYSLSSVVTVPSSSLGTQTYICNVNHKPSNTKVDKKVEPKSCDKTHTCPPCPAPEAAGGPSVFLFPPKPKDTLMISRTPEVTCVVVDVSHEDPEVKFNWYVDGVEVHNAKTKPREEQYNSTYRVVSVLTVLHQDWLNGKEYKCKVSNKALGAPIEKTISKAKGQPREPQVYTLPPCRDELTKNQVSLWCLVKGFYPSDIAVEWESNGQPENNYKTTPPVLDSDGSFFLYSKLTVDKSRWQQGNVFSCSVMHEALHNHYTQKSLSLSP

SEQ ID NO: 153 - protein, 218 aa, synthetic construct
  REGION 1..218: note = CEACAM5 VL-CL(RK)
EIVLTQSPATLSLSPGERATLSCRAGESVDIFGVGFLHWYQQKPGQAPRLLIYRASNRATGIPARFSGSGSGTDFTLTISSLEPEDFAVYYCQQTNEDPYTFGQGTKLEIKRTVAAPSVFIFPPSDRKLKSGTASVVCLLNNFYPREAKVQWKVDNALQSGNSQESVTEQDSKDSTYSLSSTLTLSKADYEKHKVYACEVTHQGLSSPVTKSFNRGEC

SEQ ID NO: 154 - protein, 5 aa, synthetic construct
  REGION 1..5: note = CEA-HCDR1
EFGMN

SEQ ID NO: 155 - protein, 17 aa, synthetic construct
  REGION 1..17: note = CEA-HCDR2
WINTKTGEATYVEEFKG

SEQ ID NO: 156 - protein, 12 aa, synthetic construct
  REGION 1..12: note = CEA-HCDR3
WDFAYYVEAMDY

SEQ ID NO: 157 - protein, 11 aa, synthetic construct
  REGION 1..11: note = CEA-LCDR1
KASAAVGTYVA

SEQ ID NO: 158 - protein, 7 aa, synthetic construct
  REGION 1..7: note = CEA-LCDR2
SASYRKR

SEQ ID NO: 159 - protein, 10 aa, synthetic construct
  REGION 1..10: note = CEA-LCDR3
HQYYTYPLFT

SEQ ID NO: 160 - protein, 121 aa, synthetic construct
  REGION 1..121: note = CEA VH
QVQLVQSGAEVKKPGASVKVSCKASGYTFTEFGMNWVRQAPGQGLEWMGWINTKTGEATYVEEFKGRVTFTTDTSTSTAYMELRSLRSDDTAVYYCARWDFAYYVEAMDYWGQGTTVTVSS

SEQ ID NO: 161 - protein, 108 aa, synthetic construct
  REGION 1..108: note = CEA VL
DIQMTQSPSSLSASVGDRVTITCKASAAVGTYVAWYQQKPGKAPKLLIYSASYRKRGVPSRFSGSGSGTDFTLTISSLQPEDFATYYCHQYYTYPLFTFGQGTKLEIK

SEQ ID NO: 162 - protein, 5 aa, synthetic construct
  REGION 1..5: note = CEA-HCDR1 (CEACAM5)
DTYMH

SEQ ID NO: 163 - protein, 17 aa, synthetic construct
  REGION 1..17: note = CEA-HCDR2 (CEACAM5)
RIDPANGNSKYVPKFQG

SEQ ID NO: 164 - protein, 12 aa, synthetic construct
  REGION 1..12: note = CEA-HCDR3 (CEACAM5)
FGYYVSDYAMAY

SEQ ID NO: 165 - protein, 15 aa, synthetic construct
  REGION 1..15: note = CEA-LCDR1 (CEACAM5)
RAGESVDIFGVGFLH

SEQ ID NO: 166 - protein, 7 aa, synthetic construct
  REGION 1..7: note = CEA-LCDR2 (CEACAM5)
RASNRAT

SEQ ID NO: 167 - protein, 9 aa, synthetic construct
  REGION 1..9: note = CEA-LCDR3 (CEACAM5)
QQTNEDPYT

SEQ ID NO: 168 - protein, 121 aa, synthetic construct
  REGION 1..121: note = CEA VH (CEACAM5)
QVQLVQSGAEVKKPGSSVKVSCKASGFNIKDTYMHWVRQAPGQGLEWMGRIDPANGNSKYVPKFQGRVTITADTSTSTAYMELSSLRSEDTAVYYCAPFGYYVSDYAMAYWGQGTLVTVSS

SEQ ID NO: 169 - protein, 111 aa, synthetic construct
  REGION 1..111: note = CEA VL (CEACAM5)
EIVLTQSPATLSLSPGERATLSCRAGESVDIFGVGFLHWYQQKPGQAPRLLIYRASNRATGIPARFSGSGSGTDFTLTISSLEPEDFAVYYCQQTNEDPYTFGQGTKLEIK